European Patent Application EP 4 606 823 A1, published August 27, 2025. Title: SYNTHETIC T CELL RECEPTOR ANTIGEN RECEPTOR SPECIFICALLY BINDING TO LILRB4 AND USE THEREOF. Applicant: BRISTAR IMMUNOTECH LIMITED. The sequence listing filed with the application follows.

SEQUENCE LISTING (123 sequences)

SEQ ID NO: 1 - protein, 141 aa, synthetic construct
DIQNPDPAVYQLRDSKSSDKSVCLFTDFDSQTNVSQSKDSDVYITDKTVLDMRSMDFKSNSAVAWSNKSDFACANAFNNSIIPEDTFFPSPESSCDVKLVEKSFETDTNLNFQNLSVIGFRILLLKVAGFNLLMTLRLWSS

SEQ ID NO: 2 - protein, 176 aa, synthetic construct
DLKNVFPPEVAVFEPSEAEISHTQKATLVCLATGFFPDHVELSWWVNGKEVHSGVSTDPQPLKEQPALNDSRYCLSSRLRVSATFWQNPRNHFRCQVQFYGLSENDEWTQDRAKPVTQIVSAEAWGRADCGFTSVSYQQGVLSATILYEILLGKATLYAVLVSALVLMAMVKRKDF

SEQ ID NO: 3 - protein, 137 aa, synthetic construct
DIQNPEPAVYQLKDPRSQDSTLCLFTDFDSQINVPKTMESGTFITDKTVLDMKAMDSKSNGAIAWSNQTSFTCQDIFKETNATYPSSDVPCDATLTEKSFETDMNLNFQNLSVMGLRILLLKVAGFNLLMTLRLWSS

SEQ ID NO: 4 - protein, 172 aa, synthetic construct
DLRNVTPPKVSLFEPSKAEIANKQKATLVCLARGFFPDHVELSWWVNGKEVHSGVSTDPQAYKESNYSYCLSSRLRVSATFWHNPRNHFRCQVQFHGLSEEDKWPEGSPKPVTQNISAEAWGRADCGITSASYQQGVLSATILYEILLGKATLYAVLVSTLVVMAMVKRKNS

SEQ ID NO: 5 - protein, 137 aa, synthetic construct
DIQNPEPAVYQLKDPRSQDSTLCLFTDFDSQINVPKTMESGTFITDKCVLDMKAMDSKSNGAIAWSNQTSFTCQDIFKETNATYPSSDVPCDATLTEKSFETDMNLNFQNLSVMGLRILLLKVAGFNLLMTLRLWSS

SEQ ID NO: 6 - protein, 172 aa, synthetic construct
DLRNVTPPKVSLFEPSKAEIANKQKATLVCLARGFFPDHVELSWWVNGKEVHSGVCTDPQAYKESNYSYCLSSRLRVSATFWHNPRNHFRCQVQFHGLSEEDKWPEGSPKPVTQNISAEAWGRADCGITSASYQQGVLSATILYEILLGKATLYAVLVSTLVVMAMVKRKNS

SEQ ID NO: 7 - protein, 137 aa, synthetic construct
DIQNPEPAVYQLKDPRSQDSTLCLFTDFDSQINVPKTMESGTFITDKTVLDMKAMDSKSNGAIAWSNQTSFTCQDIFKETNATYPSSDVPCDATLTEKSFETDMNLNFQNLLVIVLRILLLKVAGFNLLMTLRLWSS

SEQ ID NO: 8 - protein, 137 aa, synthetic construct
DIQNPEPAVYQLKDPRSQDSTLCLFTDFDSQINVPKTMESGTFITDKTVLDMKAMDSKSNGAIAWSNQTSFTCQDIFKETNATYPSSDVPCDATLTEKSFETDMNLNFQNLSVMGLRILLLRVAGFNLLMTLRLWSS

SEQ ID NO: 9 - protein, 172 aa, synthetic construct
DLRNVTPPKVSLFEPSKAEIANKQKATLVCLARGFFPDHVELSWWVNGKEVHSGVSTDPQAYKESNYSYCLSSRLRVSATFWHNPRNHFRCQVQFHGLSEEDKWPEGSPKPVTQNISAEAWGRADCGITSASYQQGVLSATILYEILLGRATLYAVLVSTLVVMAMVRRRNS

SEQ ID NO: 10 - protein, 58 aa, synthetic construct
KKVAKKPTNKAPHPKQEPQEINFPDDLPGSNTAAPVQETLHGCQPVTQEDGKESRISV

SEQ ID NO: 11 - protein, 37 aa, synthetic construct
RRDQRLPPDAHKPPGGGSFRTPIQEEQADAHSTLAKI

SEQ ID NO: 12 - protein, 34 aa, synthetic construct
KKKYSSSVHDPNGEYMFMRAVNTAKKSRLTDVTL

SEQ ID NO: 13 - protein, 41 aa, synthetic construct
RSKRSRLLHSDYMNMTPRRPGPTRKHYQPYAPPRDFAAYRS

SEQ ID NO: 14 - protein, 42 aa, synthetic construct
KRGRKKLLYIFKQPFMRPVQTTQEEDGCSCRFPEEEEGGCEL

SEQ ID NO: 15 - protein, 48 aa, synthetic construct
QRRKYRSNKGESPVEPAEPCRYSCPREEEGSTIPIQEDYRKPEPACSP

SEQ ID NO: 16 - protein, 135 aa, synthetic construct
DIQNPEPAVYQLKDPRSQDSTLCLFTDFDSQINVPKTMESGTFITDKCVLDMKAMDSKSNGAIAWSNQTSFTCQDIFKETNATYPSSDVPCDATLTEKSFETDMNLNFQNLLVIVLRILLLKVAGFNLLMTLRLW

SEQ ID NO: 17 - protein, 166 aa, synthetic construct
DLRNVTPPKVSLFEPSKAEIANKQKATLVCLARGFFPDHVELSWWVNGKEVHSGVCTDPQAYKESNYSYCLSSRLRVSATFWHNPRNHFRCQVQFHGLSEEDKWPEGSPKPVTQNISAEAWGRADCGITSASYQQGVLSATILYEILLGKATLYAVLVSTLVVMAM

SEQ ID NO: 18 - protein, 182 aa, synthetic construct
MEQGKGLAVLILAIILLQGTLAQSIKGNHLVKVYDYQEDGSVLLTCDAEAKNITWFKDGKMIGFLTEDKKKWNLGSNAKDPRGMYQCKGSQNKSKPLQVYYRMCQNCIELNAATISGFLFAEIVSIFVLAVGVYFIAGQDGVRQSRASDKQTLLPNDQLYQPLKDREDDQYSHLQGNQLRRN

SEQ ID NO: 19 - protein, 171 aa, synthetic construct
MEHSTFLSGLVLATLLSQVSPFKIPIEELEDRVFVNCNTSITWVEGTVGTLLSDITRLDLGKRILDPRGIYRCNGTDIYKDKESTVQVHYRMCQSCVELDPATVAGIIVTDVIATLLLALGVFCFAGHETGRLSGAADTQALLRNDQVYQPLRDRDDAQYSHLGGNWARNK

SEQ ID NO: 20 - protein, 207 aa, synthetic construct
MQSGTHWRVLGLCLLSVGVWGQDGNEEMGGITQTPYKVSISGTTVILTCPQYPGSEILWQHNDKNIGGDEDDKNIGSDEDHLSLKEFSELEQSGYYVCYPRGSKPEDANFYLYLRARVCENCMEMDVMSVATIVIVDICITGGLLLLVYYWSKNRKAKAKPVTRGAGAGGRQRGQNKERPPPVPNPDYEPIRKGQRDLYSGLNQRRI

SEQ ID NO: 21 - protein, 163 aa, synthetic construct
MKWKALFTAAILQAQLPITEAQSFGLLDPKLCYLLDGILFIYGVILTALFLRVKFSRSADAPAYQQGQNQLYNELNLGRREEYDVLDKRRGRDPEMGGKPRRKNPQEGLYNELQKDKMAEAYSEIGMKGERRRGKGHDGLYQGLSTATKDTYDALHMQALPPR

SEQ ID NO: 22 - protein, 94 aa, synthetic construct
NCRNTGPWLKKVLKCNTPDPSKFFSQLSSEHGGDVQKWLSSPFPSSSFSPGGLAPEISPLEVLERDKVTQLLPLNTDAYLSLQELQGQDPTHLV

SEQ ID NO: 23 - protein, 195 aa, synthetic construct
KKRIKPIVWPSLPDHKKTLEHLCKKPRKNLNVSFNPESFLDCQIHRVDDIQARDEVEGFLQDTFPQQLEESEKQRLGGDVQSPNCPSEDVVITPESFGRDSSLTCLAGNVSACDAPILSSSRSLDCRESGKNGPHVYQDLLLSLGTTNSTLPPPFSLQSGILTLNPVAQGQPILTSLGSNQEEAYVTMSSFYQNQ

SEQ ID NO: 24 - protein, 285 aa, synthetic construct
SLKTHPLWRLWKKIWAVPSPERFFMPLYKGCSGDFKKWVGAPFTGSSLELGPWSPEVPSTLEVYSCHPPRSPAKRLQLTELQEPAELVESDGVPKPSFWPTAQNSGGSAYSEERDRPYGLVSIDTVTVLDAEGPCTWPCSCEDDGYPALDLDAGLEPSPGLEDPLLDAGTTVLSCGCVSAGSPGLGGPLGSLLDRLKPPLADGEDWAGGLPWGGRSPGGVSESEAGSPLAGLDMDTFDSGFVGSDCSSPVECDFTSPGDEGPPRSYLRQWVVIPPPLSSPGPQAS

SEQ ID NO: 25 - protein, 4 aa, synthetic construct
YRHQ

SEQ ID NO: 26 - protein, 103 aa, synthetic construct
NCRNTGPWLKKVLKCNTPDPSKFFSQLSSEHGGDVQKWLSSPFPSSSFSPGGLAPEISPLEVLERDKVTQLLPLNTDAYLSLQELQGQDPTHLVGGGGSYRHQ

SEQ ID NO: 27 - protein, 204 aa, synthetic construct
KKRIKPIVWPSLPDHKKTLEHLCKKPRKNLNVSFNPESFLDCQIHRVDDIQARDEVEGFLQDTFPQQLEESEKQRLGGDVQSPNCPSEDVVITPESFGRDSSLTCLAGNVSACDAPILSSSRSLDCRESGKNGPHVYQDLLLSLGTTNSTLPPPFSLQSGILTLNPVAQGQPILTSLGSNQEEAYVTMSSFYQNQGGGGSYRHQ

SEQ ID NO: 28 - protein, 121 aa, synthetic construct
DVQLQESGGGLVQSGGSLRLSCLASGTSGNVKAVGWYGWYRQAPGKQREVVATITRGGIPNYADSVQGRFTISRDNAQDTVFLQMNSLKPADTAVYYCYARILTDDWHDLWGQGTQVTVSS

SEQ ID NO: 29 - protein, 127 aa, synthetic construct
DVQLQESGGGLVQPGGSLRLSCAASGFTLDYYAIGWFRQAPGKEREGVSCVSSSDGSTYYADSVKGRFTISRDNAKNTVYLQMNSLKPEDTAVYYCAADQYSSTWTIRLTRCHFGSWGQGTQVTVSS

SEQ ID NO: 30 - protein, 137 aa, synthetic construct
DIQNPEPAVYQLKDPRSQDSTLCLFTDFDSQINVPKTMESGTFITDKCVLDMKAMDSKSNGAIAWSNQTSFTCQDIFKETNATYPSSDVPCDATLTEKSFETDMNLNFQNLLVIVLRILLLKVAGFNLLMTLRLWSS

SEQ ID NO: 31 - protein, 133 aa, synthetic construct
DIQNPDPAVYQLRDDSTLCLFTDFDSQINVPKTMESGTFITDKCVLDMKAMDSKSNGAIAWSNQTSFTCQDIFKETNATYPSSDVPCDATLTEKSFETDMNLNFQNLLVIVLRILLLKVAGFNLLMTLRLWSS

SEQ ID NO: 32 - protein, 166 aa, synthetic construct
DLKNVFPPEVAVFEPSAEIATLVCLARGFFPDHVELSWWVNGKEVHSGVCTDPQAYKESNYSYCLSSRLRVSATFWHNPRNHFRCQVQFHGLSEEDKWPEGSPKPVTQNISAEAWGRADCGITSASYQQGVLSATILYEILLGKATLYAVLVSTLVVMAMVKRKNS

SEQ ID NO: 33 - protein, 10 aa, synthetic construct
GTSGNVKAVG

SEQ ID NO: 34 - protein, 9 aa, synthetic construct
TITRGGIPN

SEQ ID NO: 35 - protein, 10 aa, synthetic construct
RILTDDWHDL

SEQ ID NO: 36 - protein, 10 aa, synthetic construct
GFTLDYYAIG

SEQ ID NO: 37 - protein, 10 aa, synthetic construct
CVSSSDGSTY

SEQ ID NO: 38 - protein, 18 aa, synthetic construct
DQYSSTWTIRLTRCHFGS

SEQ ID NO: 39 - protein, 552 aa, synthetic construct
MLLLVTSLLLCELPHPAFLLIPDVQLQESGGGLVQSGGSLRLSCLASGTSGNVKAVGWYGWYRQAPGKQREVVATITRGGIPNYADSVQGRFTISRDNAQDTVFLQMNSLKPADTAVYYCYARILTDDWHDLWGQGTQVTVSSEDLRNVTPPKVSLFEPSKAEIANKQKATLVCLARGFFPDHVELSWWVNGKEVHSGVCTDPQAYKESNYSYCLSSRLRVSATFWHNPRNHFRCQVQFHGLSEEDKWPEGSPKPVTQNISAEAWGRADCGITSASYQQGVLSATILYEILLGKATLYAVLVSTLVVMAMVKRKNSRRKRSGSGATNFSLLKQAGDVEENPGPMLLLVTSLLLCELPHPAFLLIPDIQNPEPAVYQLKDPRSQDSTLCLFTDFDSQINVPKTMESGTFITDKCVLDMKAMDSKSNGAIAWSNQTSFTCQDIFKETNATYPSSDVPCDATLTEKSFETDMNLNFQNLLVIVLRILLLKVAGFNLLMTLRLWGGGGSGGGGSGGGGSRRDQRLPPDAHKPPGGGSFRTPIQEEQADAHSTLAKI

SEQ ID NO: 40 - protein, 558 aa, synthetic construct
MLLLVTSLLLCELPHPAFLLIPDVQLQESGGGLVQPGGSLRLSCAASGFTLDYYAIGWFRQAPGKEREGVSCVSSSDGSTYYADSVKGRFTISRDNAKNTVYLQMNSLKPEDTAVYYCAADQYSSTWTIRLTRCHFGSWGQGTQVTVSSEDLRNVTPPKVSLFEPSKAEIANKQKATLVCLARGFFPDHVELSWWVNGKEVHSGVCTDPQAYKESNYSYCLSSRLRVSATFWHNPRNHFRCQVQFHGLSEEDKWPEGSPKPVTQNISAEAWGRADCGITSASYQQGVLSATILYEILLGKATLYAVLVSTLVVMAMVKRKNSRRKRSGSGATNFSLLKQAGDVEENPGPMLLLVTSLLLCELPHPAFLLIPDIQNPEPAVYQLKDPRSQDSTLCLFTDFDSQINVPKTMESGTFITDKCVLDMKAMDSKSNGAIAWSNQTSFTCQDIFKETNATYPSSDVPCDATLTEKSFETDMNLNFQNLLVIVLRILLLKVAGFNLLMTLRLWGGGGSGGGGSGGGGSRRDQRLPPDAHKPPGGGSFRTPIQEEQADAHSTLAKI

SEQ ID NO: 41 - protein, 679 aa, synthetic construct
MLLLVTSLLLCELPHPAFLLIPDVQLQESGGGLVQSGGSLRLSCLASGTSGNVKAVGWYGWYRQAPGKQREVVATITRGGIPNYADSVQGRFTISRDNAQDTVFLQMNSLKPADTAVYYCYARILTDDWHDLWGQGTQVTVSSEDLRNVTPPKVSLFEPSKAEIANKQKATLVCLARGFFPDHVELSWWVNGKEVHSGVCTDPQAYKESNYSYCLSSRLRVSATFWHNPRNHFRCQVQFHGLSEEDKWPEGSPKPVTQNISAEAWGRADCGITSASYQQGVLSATILYEILLGKATLYAVLVSTLVVMAMVKRKNSRRKRSGSGATNFSLLKQAGDVEENPGPMLLLVTSLLLCELPHPAFLLIPDVQLQESGGGLVQPGGSLRLSCAASGFTLDYYAIGWFRQAPGKEREGVSCVSSSDGSTYYADSVKGRFTISRDNAKNTVYLQMNSLKPEDTAVYYCAADQYSSTWTIRLTRCHFGSWGQGTQVTVSSDIQNPEPAVYQLKDPRSQDSTLCLFTDFDSQINVPKTMESGTFITDKCVLDMKAMDSKSNGAIAWSNQTSFTCQDIFKETNATYPSSDVPCDATLTEKSFETDMNLNFQNLLVIVLRILLLKVAGFNLLMTLRLWGGGGSGGGGSGGGGSRRDQRLPPDAHKPPGGGSFRTPIQEEQADAHSTLAKI

SEQ ID NO: 42 - protein, 689 aa, synthetic construct
MLLLVTSLLLCELPHPAFLLIPDVQLQESGGGLVQSGGSLRLSCLASGTSGNVKAVGWYGWYRQAPGKQREVVATITRGGIPNYADSVQGRFTISRDNAQDTVFLQMNSLKPADTAVYYCYARILTDDWHDLWGQGTQVTVSSEDLRNVTPPKVSLFEPSKAEIANKQKATLVCLARGFFPDHVELSWWVNGKEVHSGVCTDPQAYKESNYSYCLSSRLRVSATFWHNPRNHFRCQVQFHGLSEEDKWPEGSPKPVTQNISAEAWGRADCGITSASYQQGVLSATILYEILLGKATLYAVLVSTLVVMAMVKRKNSRRKRSGSGATNFSLLKQAGDVEENPGPMLLLVTSLLLCELPHPAFLLIPEQKLISEEDLDVQLQESGGGLVQPGGSLRLSCAASGFTLDYYAIGWFRQAPGKEREGVSCVSSSDGSTYYADSVKGRFTISRDNAKNTVYLQMNSLKPEDTAVYYCAADQYSSTWTIRLTRCHFGSWGQGTQVTVSSDIQNPEPAVYQLKDPRSQDSTLCLFTDFDSQINVPKTMESGTFITDKCVLDMKAMDSKSNGAIAWSNQTSFTCQDIFKETNATYPSSDVPCDATLTEKSFETDMNLNFQNLLVIVLRILLLKVAGFNLLMTLRLWGGGGSGGGGSGGGGSRRDQRLPPDAHKPPGGGSFRTPIQEEQADAHSTLAKI

SEQ ID NO: 43 - protein, 131 aa, synthetic construct
DIQNPDPAVYQLRDDSTLCLFTDFDSQINVPKTMESGTFITDKCVLDMKAMDSKSNGAIAWSNQTSFTCQDIFKETNATYPSSDVPCDATLTEKSFETDMNLNFQNLLVIVLRILLLKVAGFNLLMTLRLW

SEQ ID NO: 44 - protein, 160 aa, synthetic construct
DLKNVFPPEVAVFEPSAEIATLVCLARGFFPDHVELSWWVNGKEVHSGVCTDPQAYKESNYSYCLSSRLRVSATFWHNPRNHFRCQVQFHGLSEEDKWPEGSPKPVTQNISAEAWGRADCGITSASYQQGVLSATILYEILLGKATLYAVLVSTLVVMAM

SEQ ID NO: 45 - protein, 173 aa, synthetic construct
DKQLDADVSPKPTIFLPSIAETKLQKAGTYLCLLEKFFPDVIKIHWQEKKSNTILGSQEGNTMKTNDTYMKFSWLTVPEKSLDKEHRCIVRHENNKNGVDQEIIFPPIKTDVITMDPKDNCSKDANDTLLLQLTNTSAYYMYLLLLLKSVVYFAIITCCLLRRTAFCCNGEKS

SEQ ID NO: 46 - protein, 172 aa, synthetic construct
XKRLDADISPKPTIFLPSVAETNLHKTGTYLCLLEKFFPDVIRVYWKEKDGNTILDSQEGDTLKTNDTYMKFSWLTVPERAMGKEHRCIVKHENNKGGADQEIFFPSIKKVAVSTKPTTCWQDKNDVLQLQFTITSAYYTYLLLLLKSVIYLAIISFSLLRRTSVCGNEKKS

SEQ ID NO: 47 - protein, 154 aa, synthetic construct
XSQPHTKPSVFVMKNGTNVACLVKEFYPKDIRINLVSSKKITEFDPAIVISPSGKYNAVKLGKYEDSNSVTCSVQHDNKTVHSTDFEVKTDSTDHVKPKETENTKQPSKSCHKPKAIVHTEKVNMMSLTVLGLRMLFAKTVAVNFLLTAKLFFL

SEQ ID NO: 48 - protein, 153 aa, synthetic construct
XSQPPAKPSVFIMKNGTNVACLVKDFYPKEVTISLRSSKKIVEFDPAIVISPSGKYSAVKLGQYGDSNSVTCSVQHNSETVHSTDFEPYANSFNNEKLPEPENDTQISEPCYGPRVTVHTEKVNMMSLTVLGLRLLFAKTIAINFLLTVKLFF

SEQ ID NO: 49 - protein, 5 aa, synthetic construct
EAAAK

SEQ ID NO: 50 - protein, 10 aa, synthetic construct
EAAAKEAAAK

SEQ ID NO: 51 - protein, 15 aa, synthetic construct
EAAAKEAAAKEAAAK

SEQ ID NO: 52 - protein, 4 aa, synthetic construct
EAAK

SEQ ID NO: 53 - protein, 8 aa, synthetic construct
EAAKEAAK

SEQ ID NO: 54 - protein, 13 aa, synthetic construct
EAAAKEAAKEAAK

SEQ ID NO: 55 - protein, 13 aa, synthetic construct
AAEAAAKEAAAKA

SEQ ID NO: 56 - protein, 19 aa, synthetic construct
AAAEAAAKEAAAKEAAAKA

SEQ ID NO: 57 - protein, 30 aa, synthetic construct
AAAAEAAAKEAAAKEAAAKEAAAKEAAAKA

SEQ ID NO: 58 - protein, 36 aa, synthetic construct
AAAAAEAAAKEAAAKEAAAKEAAAKEAAAKEAAAKA

SEQ ID NO: 59 - protein, 46 aa, synthetic construct
AEAAAKEAAAKEAAAKEAAAKALEAEAAAKEAAAKEAAAKEAAAKA

SEQ ID NO: 60 - protein, 6 aa, synthetic construct
GGSGGS

SEQ ID NO: 61 - protein, 12 aa, synthetic construct
GGSGGSGGSGGS

SEQ ID NO: 62 - protein, 18 aa, synthetic construct
GGSGGSGGSGGSGGSGGS

SEQ ID NO: 63 - protein, 24 aa, synthetic construct
GGSGGSGGSGGSGGSGGSGGSGGS

SEQ ID NO: 64 - protein, 30 aa, synthetic construct
GGSGGSGGSGGSGGSGGSGGSGGSGGSGGS

SEQ ID NO: 65 - protein, 36 aa, synthetic construct
GGSGGSGGSGGSGGSGGSGGSGGSGGSGGSGGSGGS

SEQ ID NO: 66 - protein, 42 aa, synthetic construct
GGSGGSGGSGGSGGSGGSGGSGGSGGSGGSGGSGGSGGSGGS

SEQ ID NO: 67 - protein, 48 aa, synthetic construct
GGSGGSGGSGGSGGSGGSGGSGGSGGSGGSGGSGGSGGSGGSGGSGGS

SEQ ID NO: 68 - protein, 54 aa, synthetic construct
GGSGGSGGSGGSGGSGGSGGSGGSGGSGGSGGSGGSGGSGGSGGSGGSGGSGGS

SEQ ID NO: 69 - protein, 60 aa, synthetic construct
GGSGGSGGSGGSGGSGGSGGSGGSGGSGGSGGSGGSGGSGGSGGSGGSGGSGGSGGSGGS

SEQ ID NO: 70 - protein, 7 aa, synthetic construct
SSSSSSS

SEQ ID NO: 71 - protein, 4 aa, synthetic construct
GGGS

SEQ ID NO: 72 - protein, 8 aa, synthetic construct
GGGSGGGS

SEQ ID NO: 73 - protein, 12 aa, synthetic construct
GGGSGGGSGGGS

SEQ ID NO: 74 - protein, 16 aa, synthetic construct
GGGSGGGSGGGSGGGS

SEQ ID NO: 75 - protein, 20 aa, synthetic construct
GGGSGGGSGGGSGGGSGGGS

SEQ ID NO: 76 - protein, 24 aa, synthetic construct
GGGSGGGSGGGSGGGSGGGSGGGS

SEQ ID NO: 77 - protein, 28 aa, synthetic construct
GGGSGGGSGGGSGGGSGGGSGGGSGGGS

SEQ ID NO: 78 - protein, 32 aa, synthetic construct
GGGSGGGSGGGSGGGSGGGSGGGSGGGSGGGS

SEQ ID NO: 79 - protein, 36 aa, synthetic construct
GGGSGGGSGGGSGGGSGGGSGGGSGGGSGGGSGGGS

SEQ ID NO: 80 - protein, 40 aa, synthetic construct
GGGSGGGSGGGSGGGSGGGSGGGSGGGSGGGSGGGSGGGS

SEQ ID NO: 81 - protein, 5 aa, synthetic construct
GGGGS

SEQ ID NO: 82 - protein, 10 aa, synthetic construct
GGGGSGGGGS

SEQ ID NO: 83 - protein, 15 aa, synthetic construct
GGGGSGGGGSGGGGS

SEQ ID NO: 84 - protein, 20 aa, synthetic construct
GGGGSGGGGSGGGGSGGGGS

SEQ ID NO: 85 - protein, 25 aa, synthetic construct
GGGGSGGGGSGGGGSGGGGSGGGGS

SEQ ID NO: 86 - protein, 30 aa, synthetic construct
GGGGSGGGGSGGGGSGGGGSGGGGSGGGGS

SEQ ID NO: 87 - protein, 35 aa, synthetic construct
GGGGSGGGGSGGGGSGGGGSGGGGSGGGGSGGGGS

SEQ ID NO: 88 - protein, 40 aa, synthetic construct
GGGGSGGGGSGGGGSGGGGSGGGGSGGGGSGGGGSGGGGS

SEQ ID NO: 89 - protein, 45 aa, synthetic construct
GGGGSGGGGSGGGGSGGGGSGGGGSGGGGSGGGGSGGGGSGGGGS

SEQ ID NO: 90 - protein, 50 aa, synthetic construct
GGGGSGGGGSGGGGSGGGGSGGGGSGGGGSGGGGSGGGGSGGGGSGGGGS

SEQ ID NO: 91 - skipped

SEQ ID NO: 92 - protein, 6 aa, synthetic construct
GGSGGS

SEQ ID NO: 93 - protein, 9 aa, synthetic construct
GGSGGSGGS

SEQ ID NO: 94 - protein, 12 aa, synthetic construct
GGSGGSGGSGGS

SEQ ID NO: 95 - protein, 15 aa, synthetic construct
GGSGGSGGSGGSGGS

SEQ ID NO: 96 - protein, 18 aa, synthetic construct
GGSGGSGGSGGSGGSGGS

SEQ ID NO: 97 - protein, 21 aa, synthetic construct
GGSGGSGGSGGSGGSGGSGGS

SEQ ID NO: 98 - protein, 24 aa, synthetic construct
GGSGGSGGSGGSGGSGGSGGSGGS

SEQ ID NO: 99 - protein, 27 aa, synthetic construct
GGSGGSGGSGGSGGSGGSGGSGGSGGS

SEQ ID NO: 100 - protein, 30 aa, synthetic construct; identical to SEQ ID NO: 64

SEQ ID NO: 101 - skipped

SEQ ID NO: 102 - protein, 4 aa, synthetic construct
GSGS

SEQ ID NO: 103 - protein, 6 aa, synthetic construct
GSGSGS

SEQ ID NO: 104 - protein, 8 aa, synthetic construct
GSGSGSGS

SEQ ID NO: 105 - protein, 10 aa, synthetic construct
GSGSGSGSGS

SEQ ID NO: 106 - protein, 12 aa, synthetic construct
GSGSGSGSGSGS

SEQ ID NO: 107 - protein, 14 aa, synthetic construct
GSGSGSGSGSGSGS

SEQ ID NO: 108 - protein, 16 aa, synthetic construct
GSGSGSGSGSGSGSGS

SEQ ID NO: 109 - protein, 18 aa, synthetic construct
GSGSGSGSGSGSGSGSGS

SEQ ID NO: 110 - protein, 20 aa, synthetic construct
GSGSGSGSGSGSGSGSGSGS

SEQ ID NO: 111 - protein, 5 aa, synthetic construct
GGGGG

SEQ ID NO: 112 - protein, 11 aa, synthetic construct
AAAAAAAAAAA

SEQ ID NO: 113 - protein, 21 aa, synthetic construct
VKQTLNFDLLKLAGCVESNPG

SEQ ID NO: 114 - protein, 22 aa, synthetic construct
GSGATNFSLLKQAGDVEENPGP

SEQ ID NO: 115 - protein, 17 aa, synthetic construct
EGRGSLLTCGDVEENPG

SEQ ID NO: 116 - protein, 19 aa, synthetic construct
QCTNYALLKLAGDVESNPG

SEQ ID NO: 117 - protein, 20 aa, synthetic construct
LEAGCKNFFPRSFTSCGSLE

SEQ ID NO: 118 - DNA, 363 bp, synthetic construct
  source 1..363: mol_type = other DNA
gatgtgcagctgcaggagagcggcggcggactggttcaatctggaggcagcctgaggctgagctgtctggccagcggaacctccggcaacgtgaaggccgtgggctggtacggctggtatagacaggcccctggcaagcagcgggaagtggtggccacaatcaccagaggcggcatccccaattacgccgatagcgtgcaaggcagattcaccatcagccgggacaacgcccaggacacagtgttcctgcagatgaacagcctgaaacctgctgataccgccgtgtactactgctacgccagaatcctgacagacgactggcacgacctgtggggccagggcacccaggtgaccgtgtccagc

SEQ ID NO: 119 - DNA, 381 bp, synthetic construct
  source 1..381: mol_type = other DNA
gacgtccagctgcaggagagcggcggaggactggttcaacctggaggcagcctgagactgagctgtgctgcttctggctttaccctggactactacgccatcggctggttcaggcaggcccctggcaaggaacgggaaggcgtgtcctgcgtgtccagcagtgatggctctacctactacgccgatagcgtgaagggcagattcaccatcagcagagacaacgccaagaataccgtgtatctgcagatgaacagcctgaaacctgaggacaccgccgtgtactactgcgccgccgaccagtacagctctacatggaccatccggctgacaagatgccacttcggcagctggggccagggcacacaggtgaccgtgtctagc

SEQ ID NO: 120 - DNA, 1659 bp, synthetic construct
  source 1..1659: mol_type = other DNA
atgcttctcctggtgacaagccttctgctctgtgagttaccacacccagcattcctcctgatcccagatgtgcagctgcaggagagcggcggcggactggttcaatctggaggcagcctgaggctgagctgtctggccagcggaacctccggcaacgtgaaggccgtgggctggtacggctggtatagacaggcccctggcaagcagcgggaagtggtggccacaatcaccagaggcggcatccccaattacgccgatagcgtgcaaggcagattcaccatcagccgggacaacgcccaggacacagtgttcctgcagatgaacagcctgaaacctgctgataccgccgtgtactactgctacgccagaatcctgacagacgactggcacgacctgtggggccagggcacccaggtgaccgtgtccagcgaggacctgagaaacgtgaccccccccaaggtgagcctgttcgagcccagcaaggccgagatcgccaacaagcagaaggccaccctggtgtgcctggccagaggcttcttccccgaccacgtggagctgagctggtgggtgaacggcaaggaggtgcacagcggcgtgtgcaccgacccccaggcctacaaggagagcaactacagctactgcctgagcagcagactgagagtgagcgccaccttctggcacaaccccagaaaccacttcagatgccaggtgcagttccacggcctgagcgaggaggacaagtggcccgagggcagccccaagcccgtgacccagaacatcagcgccgaggcctggggcagagccgactgcggcatcaccagcgccagctaccagcagggcgtgctgagcgccaccatcctgtacgagatcctgctgggcaaggccaccctgtacgccgtgctggtgagcaccctggtggtgatggccatggtgaagagaaagaacagcagaagaaagagaagcggcagcggcgccaccaacttcagcctgctgaagcaggccggcgacgtggaggagaaccccggccccatgctgctgctggtgaccagcctgctgctgtgcgagctgccccaccccgccttcctgctgatccccgacatccagaaccccgagcccgccgtgtaccagctgaaggaccccagaagccaggacagcaccctgtgcctgttcaccgacttcgacagccagatcaacgtgcccaagaccatggagagcggcaccttcatcaccgacaagtgcgtgctggacatgaaggccatggacagcaagagcaacggcgccatcgcctggagcaaccagaccagcttcacctgccaggacatcttcaaggagaccaacgccacctaccccagcagcgacgtgccctgcgacgccaccctgaccgagaagagcttcgagaccgacatgaacctgaacttccagaacctgctggtgatcgtgctgagaatcctgctgctgaaggtggccggcttcaacctgctgatgaccctgagactgtggggtggcggtggcagcggcggtggtggttccggaggcggcggttctagaagagaccagagactgccccccgacgcccacaagccccccggcggcggcagcttcagaacccccatccaggaggagcaggccgacgcccacagcaccctggccaagatctga

SEQ ID NO: 121 - DNA, 1677 bp, synthetic construct
  source 1..1677: mol_type = other DNA
atgcttctcctggtgacaagccttctgctctgtgagttaccacacccagcattcctcctgatcccagacgtccagctgcaggagagcggcggaggactggttcaacctggaggcagcctgagactgagctgtgctgcttctggctttaccctggactactacgccatcggctggttcaggcaggcccctggcaaggaacgggaaggcgtgtcctgcgtgtccagcagtgatggctctacctactacgccgatagcgtgaagggcagattcaccatcagcagagacaacgccaagaataccgtgtatctgcagatgaacagcctgaaacctgaggacaccgccgtgtactactgcgccgccgaccagtacagctctacatggaccatccggctgacaagatgccacttcggcagctggggccagggcacacaggtgaccgtgtctagcgaggacctgagaaacgtgaccccccccaaggtgagcctgttcgagcccagcaaggccgagatcgccaacaagcagaaggccaccctggtgtgcctggccagaggcttcttccccgaccacgtggagctgagctggtgggtgaacggcaaggaggtgcacagcggcgtgtgcaccgacccccaggcctacaaggagagcaactacagctactgcctgagcagcagactgagagtgagcgccaccttctggcacaaccccagaaaccacttcagatgccaggtgcagttccacggcctgagcgaggaggacaagtggcccgagggcagccccaagcccgtgacccagaacatcagcgccgaggcctggggcagagccgactgcggcatcaccagcgccagctaccagcagggcgtgctgagcgccaccatcctgtacgagatcctgctgggcaaggccaccctgtacgccgtgctggtgagcaccctggtggtgatggccatggtgaagagaaagaacagcagaagaaagagaagcggcagcggcgccaccaacttcagcctgctgaagcaggccggcgacgtggaggagaaccccggccccatgctgctgctggtgaccagcctgctgctgtgcgagctgccccaccccgccttcctgctgatccccgacatccagaaccccgagcccgccgtgtaccagctgaaggaccccagaagccaggacagcaccctgtgcctgttcaccgacttcgacagccagatcaacgtgcccaagaccatggagagcggcaccttcatcaccgacaagtgcgtgctggacatgaaggccatggacagcaagagcaacggcgccatcgcctggagcaaccagaccagcttcacctgccaggacatcttcaaggagaccaacgccacctaccccagcagcgacgtgccctgcgacgccaccctgaccgagaagagcttcgagaccgacatgaacctgaacttccagaacctgctggtgatcgtgctgagaatcctgctgctgaaggtggccggcttcaacctgctgatgaccctgagactgtggggtggcggtggcagcggcggtggtggttccggaggcggcggttctagaagagaccagagactgccccccgacgcccacaagccccccggcggcggcagcttcagaacccccatccaggaggagcaggccgacgcccacagcaccctggccaagatctga

SEQ ID NO: 122 - DNA, 2040 bp, synthetic construct
  source 1..2040: mol_type = other DNA
atgcttctcctggtgacaagccttctgctctgtgagttaccacacccagcattcctcctgatcccagatgtgcagctgcaggagagcggcggcggactggttcaatctggaggcagcctgaggctgagctgtctggccagcggaacctccggcaacgtgaaggccgtgggctggtacggctggtatagacaggcccctggcaagcagcgggaagtggtggccacaatcaccagaggcggcatccccaattacgccgatagcgtgcaaggcagattcaccatcagccgggacaacgcccaggacacagtgttcctgcagatgaacagcctgaaacctgctgataccgccgtgtactactgctacgccagaatcctgacagacgactggcacgacctgtggggccagggcacccaggtgaccgtgtccagcgaggacctgagaaacgtgaccccccccaaggtgagcctgttcgagcccagcaaggccgagatcgccaacaagcagaaggccaccctggtgtgcctggccagaggcttcttccccgaccacgtggagctgagctggtgggtgaacggcaaggaggtgcacagcggcgtgtgcaccgacccccaggcctacaaggagagcaactacagctactgcctgagcagcagactgagagtgagcgccaccttctggcacaaccccagaaaccacttcagatgccaggtgcagttccacggcctgagcgaggaggacaagtggcccgagggcagccccaagcccgtgacccagaacatcagcgccgaggcctggggcagagccgactgcggcatcaccagcgccagctaccagcagggcgtgctgagcgccaccatcctgtacgagatcctgctgggcaaggccaccctgtacgccgtgctggtgagcaccctggtggtgatggccatggtgaagagaaagaacagcagaagaaagagaagcggcagcggcgccaccaacttcagcctgctgaagcaggccggcgacgtggaggagaaccccggccccatgctgctgctggtgaccagcctgctgctgtgcgagctgccccaccccgccttcctgctgatccccgacgtccagctgcaggagagcggcggaggactggttcaacctggaggcagcctgagactgagctgtgctgcttctggctttaccctggactactacgccatcggctggttcaggcaggcccctggcaaggaacgggaaggcgtgtcctgcgtgtccagcagtgatggctctacctactacgccgatagcgtgaagggcagattcaccatcagcagagacaacgccaagaataccgtgtatctgcagatgaacagcctgaaacctgaggacaccgccgtgtactactgcgccgccgaccagtacagctctacatggaccatccggctgacaagatgccacttcggcagctggggccagggcacacaggtgaccgtgtctagcgacatccagaaccccgagcccgccgtgtaccagctgaaggaccccagaagccaggacagcaccctgtgcctgttcaccgacttcgacagccagatcaacgtgcccaagaccatggagagcggcaccttcatcaccgacaagtgcgtgctggacatgaaggccatggacagcaagagcaacggcgccatcgcctggagcaaccagaccagcttcacctgccaggacatcttcaaggagaccaacgccacctaccccagcagcgacgtgccctgcgacgccaccctgaccgagaagagcttcgagaccgacatgaacctgaacttccagaacctgctggtgatcgtgctgagaatcctgctgctgaaggtggccggcttcaacctgctgatgaccctgagactgtggggtggcggtggcagcggcggtggtggttccggaggcggcggttctagaagagaccagagactgccccccgacgcccacaagccccccggcggcggcagcttcagaacccccatccaggaggagcaggccgacgcccacagcaccctggccaagatctga

SEQ ID NO: 123 - DNA, 2070 bp, synthetic construct
  source 1..2070: mol_type = other DNA
atgcttctcctggtgacaagccttctgctctgtgagttaccacacccagcattcctcctgatcccagatgtgcagctgcaggagagcggcggcggactggttcaatctggaggcagcctgaggctgagctgtctggccagcggaacctccggcaacgtgaaggccgtgggctggtacggctggtatagacaggcccctggcaagcagcgggaagtggtggccacaatcaccagaggcggcatccccaattacgccgatagcgtgcaaggcagattcaccatcagccgggacaacgcccaggacacagtgttcctgcagatgaacagcctgaaacctgctgataccgccgtgtactactgctacgccagaatcctgacagacgactggcacgacctgtggggccagggcacccaggtgaccgtgtccagcgaggacctgagaaacgtgaccccccccaaggtgagcctgttcgagcccagcaaggccgagatcgccaacaagcagaaggccaccctggtgtgcctggccagaggcttcttccccgaccacgtggagctgagctggtgggtgaacggcaaggaggtgcacagcggcgtgtgcaccgacccccaggcctacaaggagagcaactacagctactgcctgagcagcagactgagagtgagcgccaccttctggcacaaccccagaaaccacttcagatgccaggtgcagttccacggcctgagcgaggaggacaagtggcccgagggcagccccaagcccgtgacccagaacatcagcgccgaggcctggggcagagccgactgcggcatcaccagcgccagctaccagcagggcgtgctgagcgccaccatcctgtacgagatcctgctgggcaaggccaccctgtacgccgtgctggtgagcaccctggtggtgatggccatggtgaagagaaagaacagcagaagaaagagaagcggcagcggcgccaccaacttcagcctgctgaagcaggccggcgacgtggaggagaaccccggccccatgctgctgctggtgaccagcctgctgctgtgcgagctgccccaccccgccttcctgctgatccccgagcagaaactcatctctgaagaggatctggacgtccagctgcaggagagcggcggaggactggttcaacctggaggcagcctgagactgagctgtgctgcttctggctttaccctggactactacgccatcggctggttcaggcaggcccctggcaaggaacgggaaggcgtgtcctgcgtgtccagcagtgatggctctacctactacgccgatagcgtgaagggcagattcaccatcagcagagacaacgccaagaataccgtgtatctgcagatgaacagcctgaaacctgaggacaccgccgtgtactactgcgccgccgaccagtacagctctacatggaccatccggctgacaagatgccacttcggcagctggggccagggcacacaggtgaccgtgtctagcgacatccagaaccccgagcccgccgtgtaccagctgaaggaccccagaagccaggacagcaccctgtgcctgttcaccgacttcgacagccagatcaacgtgcccaagaccatggagagcggcaccttcatcaccgacaagtgcgtgctggacatgaaggccatggacagcaagagcaacggcgccatcgcctggagcaaccagaccagcttcacctgccaggacatcttcaaggagaccaacgccacctaccccagcagcgacgtgccctgcgacgccaccctgaccgagaagagcttcgagaccgacatgaacctgaacttccagaacctgctggtgatcgtgctgagaatcctgctgctgaaggtggccggcttcaacctgctgatgaccctgagactgtggggtggcggtggcagcggcggtggtggttccggaggcggcggttctagaagagaccagagactgccccccgacgcccacaagccccccggcggcggcagcttcagaacccccatccaggaggagcaggccgacgcccacagcaccctggccaagatctga